European Patent Specification EP 3 333 266 B1, published April 24, 2024. Title: A method of manufacturing selenoneine. Applicant: KIKKOMAN CORPORATION. The sequence listing filed with the application follows.

SEQUENCE LISTING (32 sequences)

SEQ ID NO: 1 - DNA, 2925 bp, Aspergillus sojae
atgtcacctttggctctctctcctaagaccgttgacattgtcaacatctttcagaatgatgtggagttctccctcgtaaatgagatccataagggtattagtcctcccgctggcgttaggaagtcaatgccaacgatgcttctttacgatgccaatggcctcaagctttttgagaacatcacctatgtgaaggagtattatctaacaaatgcggaaattgaggtcttggagacaaattccaggaggatagttgaacggattccagacaatgcgcaactgcttgaattaggtagcgggtgcgtcatccttccaaatcaaatcgtaacctttcaggctgcgtagcgtatcattaccgttctccggttttaaccgccttttaggaatcttcggaaaattgagattctgctacgggagtttgagcgcgtgggaaagcgcgtggattattatgccctggacctgtctctatcagaactgcagcgcacattcgcagaggtgtccattgatgattacacacacgttggcctccatggtctccatggaacctacgatgatgccgtcacttggcttaacagccccgaaaacaggaagcggcccacggtgatcatgtctatgggttcctctttagggaactttgaccgtcccggcgcagcaaagtttctctcgcagtatgctagccttcttggtccatccgatatgatgatcattggtctggatggctgcaaggacccgggcaaagtatacagggcatacaatgattcagaaggtgttacacggcagttctacgagaacggactagtgcatgcaaatgttgttcttggatacgaagccttcaaatctgatgagtgggaagtagtgactgactacgataccgtggagggacgacactgggcagcctactcacccaagaaggacgtcactatcaacggggtccttcttaagaagggtgagaaacttttctttgaagaggcgtacaagtacggaccagaggaacgcgatcaactgtggcgtgatgccaagttaattcagtctacggaaatgggcaatgggtctgacgattaccgtgagtagcaaatggctgcctcatttcaatagacgtgtatgctgactctggcttttcgcaaaatagatctccatcttctgacatcggctaccctcaacctccccacgtctccctctcaatatgcagctcatcctatacccagctttgaagaatggcagtccctgtggacagcatgggataatgctacaaaggctatggtccctcgcgaggagcttctgtcaaagccgatcaagctacggaactctttgatcttctatctgggacacattcctacattcttgggttagtctacatggcttactattcccaacacatagcttgatgctaattatgcaaacagacatccatctgacccgagccctgcgcggaaaattaacagagccaaagtcttataaactaattttcgaacgtgggattgatcctgatgtagatgaccccgagaagtgccactcccatagcgagatcccagacgagtggccagctcttgatgacattctagactaccaagagcgagtcagaagcagagttagatccatctaccaaatcgagggccttgcagagaacagaatcctgggtgaggcgctttggattggatttgagcacgaagtgatgcacctcgagacattcctgtacatgttgatccagagcgaaaggatacttcccccgcccgccactgagcggccggacttcaaaaaactgtatcaagaagctcggagaagcatgaaagcaaatgagtggttctctgttcctgaacagacacttactattggccttgatggtgctgataccaacgacgtacccccaacgacctatgggtgggacaatgagaaacctgcgagaacagtcacggttccagcatttgaggcgcagggcaggcccatcaccaatggtgagtacgccaagtacttgcaagcgaatcagtcgcgcagaaggccagcatcatgggtcctgacccattcggatgaagactacgccatacctatggcggtcaacggaagcagtgtcggggctacgcaggactttatgtccaactttgctgtccgtacggtcttcggcccagttccacttgaatttgctcaggactggcctgtgatggcgtcatatgatgaattagctgaatacgccgaatgggtgggttgcaggatcccaaccttcgaagagacaaggagtatctatctgcactcagcgctattgaaggaaagaggtggcgtgaatcataatggggagcccaacggccataggttagtgcagcctcattataacaccacattcgggattaagctgagctaacggctgtcagtttgaacggcgatctgaatggggtgaatggaaatggttactcgaagatcaacccaggcaaacctcgtaagccggatcaccagcctgtacaatatccttcccgagacgccctgccagtgttccttgatctgcacggtctcaacgtcgggttcaagcactggcaccccaccccagttatccagaacggcgatcgactcgccggtcagggtgaactgggaggcgcatgggagtggactagcacgccattagcgccacacgatggctttaaagccatggagatctacccgggatacacctgtaagtaccagtcccgttatcgggtaccctctaaaagtctatcattacatactaattccgcacagccgatttcttcgacggtaaacataatatcatcctgggtggttcttgggctactcatccccgcgtcgctgggcgtaccactttgtaagtttaccggtatagaactcggggcactataagatgctgacatcacctctagcgtcaattggtaccagcacaactatccttacacctgggcaggagcacgcctggtgcgggatctttag

SEQ ID NO: 2 - DNA, 1770 bp, Aspergillus sojae
atgtctaatgttacccaatcagccttgagacaggcaactcgcgcctacgctcgccgactgccatcgacgcagcatggctccttcgcttccgcccttcccagacgggcgctcgccactccatacagacggttctatgtctccgaaactaaggctggaaatgctcaggtttcggtagataccgctatgaagcaggagcagaaggaattcatgaaacaaactggggtgcagccgcagaaggtggagctccctagttctggtgtttccggcgatgcctcgatgagcccgtctgccggcatcctcaagcaggccactgtcatggaccaaggaacgcgaccgatctatctcgatatgcaggccacaaccccaacggatccccgtgttctcgacgccatgctccccttcttgaccggaatttacggcaaccctcattcgagaacccatgcatacggttgggagtcagaaaaggcagtcgagcaatcccgagagcatatcgccaagctgatcggcgcggacccgaaagagatcatcttcactagcggtgctactgagagtaacaacatgagcattaagggtgtggcgaggttttttgggcgctccggcaaaaaaaaccacatcatcacaacgcagaccgagcacaagtgtgttcttgacagctgtcggcatcttcaggatgagggctacgaggttacgtatctccccgtgcagaacaacggcttgattcggatggaagacctcgaggccgccattcgccctgaaacggccctggtcagcatcatggccgtcaacaatgagatcggtgttatccagcccctggaacagattggaaagttgtgccgctccaagaagattttcttccacacggacgctgcacaggccgtgggaaagatcccgttggatgtgaataaattgaatattgatttgatgtctatttcgagccacaagatttacggccccaagggtattggagcttgctatgtcagacgtcgtcccagggttcgccttgaccctctcattactggaggtggacaggagcgaggcctgcgcagtggtactcttgctcctcatctggtcgttgggttcggtgaggcctgccggatcgccgcccaagatatggaggtacgttctatttttcttttgtttctgcttacttgcaatcccttttctattttccgatgattatatactgcaaatatggatttccgagaccggtgggggtagctgcacgcctaacgcgtgacccatgggcctatgacgtctcagcaggggtgatgagttgactattgctttgtttgccttgtttgcctcatgcggctatgcgtcagtggacatcgctaatcgagttggcagtatgacaccaagcacattgatcgtttgtccaagcgcctgaccgacgggctcctatccatggagcacacacacctcaacggagaccctgaacatcactacccgggatgtgtcaatgtctcctttgcctacatcgaaggagagtctctcctgatggccttgaaagacattgctctgtcgtcgggtagtgcctgtacctctgcgtcattggagcccagctacgtccttcgtgccttgggtagcagtgacgagagcgcccatagcagtatccggtttggaattggacgattcacttcggatagcgaaattgactacgtgctgaaggcggtacaggaccgcgttcatttcctacgcgagctgagccccttgtgggaattggtgcaggaaggtatcgacctgaacacgatcgaatggagtcaacattaa

SEQ ID NO: 3 - DNA, 1529 bp, Aspergillus sojae
atgaccactcccttcggagctcccatgagagagcacttcctctttgacaccaacttcaaaaacctcaaccatggtatagtatcctactccagtaacaagtaccaacattagctaactataaaccaggctccttcggcacatacccccgtgccgtccagacagtcctccgccaacaccaacactccgccgaggcccgtccagacctcttctaccgcatcacccgcggccaaggcatcgacggatcgcgccgcatcgtagccaacctgctcaacatccccgtcaacgaatgtgtcttcgtcaagaacgcaaccacgggggtcgccaccgtgctccgtaatctagtcttccagaagggagacgcagtcgtgtacttcgacactatctatggcgctgtggagaagaatgtacactctattatggaggctagtcctgtgactactcgaaaggttgagtgtgcgttacccgttagccatgaggacctggtgaaacggttcagggatgtcgtgagtcgtgcaagaggggaagggctgcatgtgaaagttgcggtgtttgacaccatcgtcagtgtgcctggggtcaggttcccgttcgagaccttggtaggggtctgtcgggaggagggtatactcagtcttatcgatggggcgcatggtattggacatataccgttggatttggggactttgaggccggatttctttactagtaacctgcataagtatgttcctttcccctttctttctttctttcgtttgattactgtgtgaggatcttgtatgctgatatagagcaaaaaaaaaagatggctattcgtcccccgcggctgcgcagttctccacgtcccactccgcaaccaacatctcatccgcaccacattcccaacctcatggggatacatcccccctccctcatccggggagataacccccaccgccacgcagggtaaatccgccttcgaatatctcttcgaacacatctccacaaccgacgacacgccctggctatgcgtccccgccgccatgaaattccgaactgaagtctgcggcggcgaagaccgcatctacgcttacctggagaccctagcccgcgaggccggggatatcgttgcccgcgccctcgggacggaagtcatgcaggagcccgggttgaaggagggagaggtgagtcagcttaggaggtgtgggatggctactgtgcggttgccgattgctgtgacttcttcttcttcttctgattctgggtctggtaatggtgggggtgctgttatgagggtgcagggtgaggatgggagttcgtatttgcgaatccagacgtctttggtggggactgtgagtaattggtttcgggatacgttgtttgataagtacgagacgtttgtgccggtgttccagcatggggggtggttgtggacgagactcagtgcgcaggtttatttggagaagggggattttgagtggttggggggtgttttgagggagtgttgtgagagggttgagagggaggttggggtttcttctgcgaagctttga

SEQ ID NO: 4 - protein, 845 aa, Aspergillus sojae
MSPLALSPKTVDIVNIFQNDVEFSLVNEIHKGISPPAGVRKSMPTMLLYDANGLKLFENITYVKEYYLTNAEIEVLETNSRRIVERIPDNAQLLELGSGNLRKIEILLREFERVGKRVDYYALDLSLSELQRTFAEVSIDDYTHVGLHGLHGTYDDAVTWLNSPENRKRPTVIMSMGSSLGNFDRPGAAKFLSQYASLLGPSDMMIIGLDGCKDPGKVYRAYNDSEGVTRQFYENGLVHANVVLGYEAFKSDEWEVVTDYDTVEGRHWAAYSPKKDVTINGVLLKKGEKLFFEEAYKYGPEERDQLWRDAKLIQSTEMGNGSDDYHLHLLTSATLNLPTSPSQYAAHPIPSFEEWQSLWTAWDNATKAMVPREELLSKPIKLRNSLIFYLGHIPTFLDIHLTRALRGKLTEPKSYKLIFERGIDPDVDDPEKCHSHSEIPDEWPALDDILDYQERVRSRVRSIYQIEGLAENRILGEALWIGFEHEVMHLETFLYMLIQSERILPPPATERPDFKKLYQEARRSMKANEWFSVPEQTLTIGLDGADTNDVPPTTYGWDNEKPARTVTVPAFEAQGRPITNGEYAKYLQANQSRRRPASWVLTHSDEDYAIPMAVNGSSVGATQDFMSNFAVRTVFGPVPLEFAQDWPVMASYDELAEYAEWVGCRIPTFEETRSIYLHSALLKERGGVNHNGEPNGHSLNGDLNGVNGNGYSKINPGKPRKPDHQPVQYPSRDALPVFLDLHGLNVGFKHWHPTPVIQNGDRLAGQGELGGAWEWTSTPLAPHDGFKAMEIYPGYTSDFFDGKHNIILGGSWATHPRVAGRTTFVNWYQHNYPYTWAGARLVRDL

SEQ ID NO: 5 - protein, 512 aa, Aspergillus sojae
MSNVTQSALRQATRAYARRLPSTQHGSFASALPRRALATPYRRFYVSETKAGNAQVSVDTAMKQEQKEFMKQTGVQPQKVELPSSGVSGDASMSPSAGILKQATVMDQGTRPIYLDMQATTPTDPRVLDAMLPFLTGIYGNPHSRTHAYGWESEKAVEQSREHIAKLIGADPKEIIFTSGATESNNMSIKGVARFFGRSGKKNHIITTQTEHKCVLDSCRHLQDEGYEVTYLPVQNNGLIRMEDLEAAIRPETALVSIMAVNNEIGVIQPLEQIGKLCRSKKIFFHTDAAQAVGKIPLDVNKLNIDLMSISSHKIYGPKGIGACYVRRRPRVRLDPLITGGGQERGLRSGTLAPHLVVGFGEACRIAAQDMEYDTKHIDRLSKRLTDGLLSMEHTHLNGDPEHHYPGCVNVSFAYIEGESLLMALKDIALSSGSACTSASLEPSYVLRALGSSDESAHSSIRFGIGRFTSDSEIDYVLKAVQDRVHFLRELSPLWELVQEGIDLNTIEWSQH

SEQ ID NO: 6 - protein, 463 aa, Aspergillus sojae
MTTPFGAPMREHFLFDTNFKNLNHGSFGTYPRAVQTVLRQHQHSAEARPDLFYRITRGQGIDGSRRIVANLLNIPVNECVFVKNATTGVATVLRNLVFQKGDAVVYFDTIYGAVEKNVHSIMEASPVTTRKVECALPVSHEDLVKRFRDVVSRARGEGLHVKVAVFDTIVSVPGVRFPFETLVGVCREEGILSLIDGAHGIGHIPLDLGTLRPDFFTSNLHKWLFVPRGCAVLHVPLRNQHLIRTTFPTSWGYIPPPSSGEITPTATQGKSAFEYLFEHISTTDDTPWLCVPAAMKFRTEVCGGEDRIYAYLETLAREAGDIVARALGTEVMQEPGLKEGEVSQLRRCGMATVRLPIAVTSSSSSDSGSGNGGGAVMRVQGEDGSSYLRIQTSLVGTVSNWFRDTLFDKYETFVPVFQHGGWLWTRLSAQVYLEKGDFEWLGGVLRECCERVEREVGVSSAKL

SEQ ID NO: 7 - DNA, 748 bp, Aspergillus sojae
tgtggaccagacaggcgccactcggccgggccacaactgcttgggttttgaccgggagcggaccaattaaggactcgaacgaccgcggggttcaaatgcaaacaagtacaacacgcagcaaacgaagcagcccaccactgcgttgatgcccagtttgtctgtccgaaatccaccggaaaggtggaaacatactatgtaacaatcagagggaagaaaaattttttatcgacgaggcaggatagtgactgatggtggggtcatggtcgggtctccgagcgaaagagaaccaaggaaacaagatcaacgaggttggtgtacccaaaaggccgcagcaacaagagtcatcgcccaaaagtcaacagtctggaagagactccgccgtgcagattctgcgtcggtcccgcacatgcgtggtgggggcattacccctccatgtccaatgataagggcggcggtcgagggcttaagcccgcccactaattcgccttctcgcttgcccctccatataaggattcccctccttcccctcccacaacttttttcctctttctctcttcgtccgcatcagtacgtatatctttcccccctacctctttctcactcttcctcgattcattccactcttctccttactgacatctgttttgctcagtacctctacgcgatcagccgtagtatctgagcaagcttttttacagaatctttctagtatcttacaaagaactacaaagttcgcaccaccttcaaa

SEQ ID NO: 8 - DNA, 800 bp, Aspergillus sojae
gtaccaggagtacattggagagttctaccattgttgctggaatacaatgatgattagaaaccgaagagtgttatgattcggacggatatacgcatggcacgcatacagcgtgatacataggctgtttgctcaagaattaggattttatctgaatccatgtacagagtttacttatgttagtagtcaatgaaatcttggctttctaattttgtccgatctacaaggggtagtcgatcacagaacgaactagatgtgcagggaacgatgatcacccgctcttagcaagacctctagtagttttcgaccatagctttaacgcgaatcatgaccctactattttctagattgcagaccaagtcacatgacaatgtcctctttgaagtaggatcagtagctgattagattccgggaaatgaattagggctggcgttccaactactggggagtgccgatgttgctgtatgaaagatagtaagattactagtgcacagctgtagtaattatttactctagattatatattccaaataataagtaatctaagatagtagacagtcctatgatatagctccgggttcgaagtcggcaaaagatatgcaatcacctgtcgggatgatatatgtatatctgaaataccgacatcaaccatccagtcggatcagctaaacgaagtatcacttctttcgccactgccaatcactacttctattaaagttcatgttacagtataagccacaagacttatctccagaactaacttgtgcataggagctctgccgatagccgggtggttggatcgg

SEQ ID NO: 9 - DNA, 1838 bp, Aspergillus sojae
ttgggcttattgctatgtccctgaaaggatatcaaaagcaggcaaaaagccaggcataaccccgcgcggatggtaccctaaggataagccctaatcttatctacatgtgactgcgtcgatgtgtttggtccaaatgaggcatgtggctcaccccacaggcggagaaacgtgtggctagtgcatgacggtcccctccatagattcaatttaatttttcgcggcaattgtcgtgcagtttgtatctaccgttcattctacatattaagggttagtaattggacatcctgattactttgtctaattactgaaaactcgaagtactaacctactaaataagtcagtttcaaccactaagtactcatttatacaatagttgcagaaccccgcgctacccctccattgccaacatgtcttccaagtcgcaattgacctacagcgcacgcgctagcaagcaccccaatgcgctcgtgaagaagctcttcgaggttgccgaggccaagaaaaccaatgtcaccgtttccgccgacgtgacaaccaccaaagagctgctggatttggctgaccgtatgcgcaccggggatgccacttacatatgatctagtaatggttaatggtggaatatataacaggactcggtccgtacattgccgtgatcaaaactcacatcgatatcctctccgatttcagcgaagagaccatcatcggtctgaaggcccttgcagagaagcacaatttcctcatcttcgaagatcgcaagttcatcgatatcggaaacacagtccaaaagcagtaccatggcggcactctgcgcatctctgagtgggcccacatcatcaactgcagtattctgcccggtgagggtatcgtcgaggctctggcccagactgcttcggccgaggacttcccctatggctctgagaggggccttttgatccttgcggagatgacatccaagggatctttggctaccggtcaatatactacttcttctgttgactatgcccggaagtataagaagtttgtgatgggattcgtctcgacgcgtcacctgggcgaggttcagtctgaagttagctcgccttcggaggaggaggatttcgtcgtcttcacgacaggtgtcaacctctcctcgaagggagacaaactgggacagcaataccagactcctgagtctgctgttggacgcggtgccgactttatcattgctggtcgtggaatttatgctgctcctgatcccgtggaggcagcgaagcggtaccagaaagagggatgggatgcataccagaagcgtgttggtgcgcaataagtagtggtgaatacgtgctctttttatggcagtatatcgcaagtatgatgcgattcataaattcagcagtcgaattctacgagagaacgatgctaagagataccctctctatatgaataatatgcctgcctcgagatatggacatattcaagatcagagttaagggtcatgtttcaaaatcacaccaatctccaacatagacgagaatttttaccggattgtctgaaggtgcagctggagattggtctattttctaagagtggggtatcactaatgtacagtcggtcactatcgtacaaacaatcacaattatatacaagatttcccatcaccccttactctaacatggcacttttatccatcgagtccgagcctagccaccatttggtgctttcgtagagaccaaagtataaccctgatccgacagcggccataaacgtgttgatagcacaccctcggaatagtcctctcgggccatctgttcgtataatctcccgtacggtattgatcatccttttcttctgaggtgcgg

SEQ ID NO: 10 - DNA, 38 bp, Artificial sequence
  Primer
cggtacccggggatctgtggaccagacaggcgccactc

SEQ ID NO: 11 - DNA, 40 bp, Artificial sequence
  Primer
atgtactcctggtactttgaaggtggtgcgaactttgtag

SEQ ID NO: 12 - DNA, 28 bp, Artificial sequence
  Primer
gtaccaggagtacattggagagttctac

SEQ ID NO: 13 - DNA, 23 bp, Artificial sequence
  Primer
ccgatccaaccacccggctatcg

SEQ ID NO: 14 - DNA, 43 bp, Artificial sequence
  Primer
gggtggttggatcggttgggcttattgctatgtccctgaaagg

SEQ ID NO: 15 - DNA, 39 bp, Artificial sequence
  Primer
cgactctagaggatcccgcacctcagaagaaaaggatga

SEQ ID NO: 16 - DNA, 25 bp, Artificial sequence
  Primer
tttgaaggtggtgcgaactttgtag

SEQ ID NO: 17 - DNA, 38 bp, Artificial sequence
  Primer
cgcaccaccttcaaaatgtcacctttggctctctctcc

SEQ ID NO: 18 - DNA, 37 bp, Artificial sequence
  Primer
atgtactcctggtacctaaagatcccgcaccaggcgt

SEQ ID NO: 19 - DNA, 44 bp, Artificial sequence
  Primer
cgcaccaccttcaaaatgtctaatgttacccaatcagccttgag

SEQ ID NO: 20 - DNA, 45 bp, Artificial sequence
  Primer
atgtactcctggtacttaatgttgactccattcgatcgtgttcag

SEQ ID NO: 21 - DNA, 36 bp, Artificial sequence
  Primer
cgcaccaccttcaaaatgaccactcccttcggagct

SEQ ID NO: 22 - DNA, 43 bp, Artificial sequence
  Primer
atgtactcctggtactcaaagcttcgcagaagaaaccccaacc

SEQ ID NO: 23 - DNA, 2917 bp, Aspergillus oryzae
atgtcaccgttggctctttctcctaagaccgttgacattgtcaacatctttcagaatgacgtggagttctccctcgtaaatgagatccataagggcattagtcctcccgctggcgttaggaagtcaatgccaacgatgcttctttacgatgccaatggcctcaagctttttgagaaaatcacctatgtgaaggagtattatctaacaaatgcggaaatcgaggtcttggagacaaattccaggaggatagttgaacggattccagacaatgcgcaactgcttgaattaggtagcgggtgcgtcatccttccaaatcaaatcgtaacctttcaggctgcgtagcgtatcattaccgttctccggttttaaccgccttttaggaatcttcggaaaattgagattctgctacgggagtttgagcgcgtgggaaagcgcgtggattattatgcccttgacctgtctctatcagaactgcagcgcacattcgcagaggtgtccattgatgattacacacacgttggcctccatggtctccatggaacctacgacgatgccgtcacttggcttaacagccccgaaaacaggaagcggcccacggtgatcatgtctatgggttcctctttagggaactttgaccgtcctggcgcagcaaagtttctctcgcagtatgctagccttcttggtccatccgatatgatgatcattggtctggatggctgcaaggacccgggcaaagtatacagggcatacaatgattcagaaggtgttacacggcagttctatgagaacggactagtgcatgcaaatgttgttcttggatacgaagccttcaaacctgatgagtgggaagtagtgactgactacgatgccgtggagggacgacactgggcagcctactcacccaggagggacgtcactatcaacggggtccttcttaagaagggggagaaactcttctttgaagaggcgtacaagtacggaccagaggaacgcgatcaactgtggcgtgatgccaagttactccagtctacggaagtgggcaatgggtctgacgattaccgtgagtagcaaatggctgcctcatttcagtagacgtgtatgctaaatctggcttttcgcaaaatagatctccatcttctgacatccgctgccctcaacctccccacgtctccctctcaatatgcagctcatcctatacccagctttgaagaatggcagtccctgtggacagcatgggataatgctacaaaggctatggtccctcgcgaggagcttctgtcaaagccgatcaagctacggaactctttaatcttctatctggggcacattcctacattcttgggttagtctacatggcttactattcccaacacataacttgatgctaattatgcaaacagacatccatctgacccgagccctgcgcggaaaactgacagagccaaagtcttataaactaattttcgaacgtgggattgatcctgatgtagatgacccccagaagtgccactcccatagcgagatcccagacgagtggccagctcttgatgacattctagactaccaagagcgagtcagaagcagagttagatccatctaccagatcgagggccttgcagaaaacagaatcctgggtgaggcgctttggattggatttgagcacgaagtgatgcacctcgagacattcctgtacatgttgatccagagcgaaaggatacttcccccgcccgccactgaacggccggacttcaaaaaactgtaccaagacgctcggagaagcatgaaaacaaatgagtggttctccgttcctgaacagacacttactattggccttgatggtgctgataccaacgacgtacccccaacgacctatgggtgggacaatgagaaacctgcgagaacagtgacggttccagcatttgaggcgcagggcaggcccatcaccaatggtgagtacgccaagtacttgcaagcgaatcagtcgcgcagaaggccagcatcatgggtcctgacccattcggatgaaaactaccccatacctatggccgtcaacggaagcagtgtcggggctacgcaggactttatgtccaactttgctgtccgtactgtcttcggcccagttccacttgaatttgctcaggactggcctgtgatggcgtcatatgatgaattagccgaatatgccgaatgggtgggttgcagaatcccaaccttcgaagagacaaggagtatctatctgcactcagcgctactgaaggaaagaggtggcgtaaatcataatggggagcccaatggccataggttagtgcagcctcattataacgccacattccggggattgagctgagctaacggctttcagtgtgaacggctatctgaacgggatgaatggaaatagctactcgaagatcaacccaggcaaacctcgtacgccggaccaccagcctgtacaatatccttcccgggacgccttgccagtgttccttgatctggacggtctcaacgtcgggttcaagcactggcaccccaccccagttatccagaacggcgatcgactcgccggtcagggtgaactgggaggcgcatgggagtggactagcacgccattagcgccacacgatggctttaaagccatggagatctacccgggatacacctgtaagtaccagtcccgttatcgggtaccctctcattacatactaattccgcacagccgatttcttcgacggtaaacataacatcatcctgggtggttcttgggctactcatccccgcgttgctgggcgtaccactttgtaagtttaccggtatagaacccggggcactataagatgctgacaacacctctagcgtcaattggtaccagcacaactatccttacacctgggcaggagcacgcctagtgcgggatctttag

SEQ ID NO: 24 - protein, 845 aa, Aspergillus oryzae
MSPLALSPKTVDIVNIFQNDVEFSLVNEIHKGISPPAGVRKSMPTMLLYDANGLKLFEKITYVKEYYLTNAEIEVLETNSRRIVERIPDNAQLLELGSGNLRKIEILLREFERVGKRVDYYALDLSLSELQRTFAEVSIDDYTHVGLHGLHGTYDDAVTWLNSPENRKRPTVIMSMGSSLGNFDRPGAAKFLSQYASLLGPSDMMIIGLDGCKDPGKVYRAYNDSEGVTRQFYENGLVHANVVLGYEAFKPDEWEVVTDYDAVEGRHWAAYSPRRDVTINGVLLKKGEKLFFEEAYKYGPEERDQLWRDAKLLQSTEVGNGSDDYHLHLLTSAALNLPTSPSQYAAHPIPSFEEWQSLWTAWDNATKAMVPREELLSKPIKLRNSLIFYLGHIPTFLDIHLTRALRGKLTEPKSYKLIFERGIDPDVDDPQKCHSHSEIPDEWPALDDILDYQERVRSRVRSIYQIEGLAENRILGEALWIGFEHEVMHLETFLYMLIQSERILPPPATERPDFKKLYQDARRSMKTNEWFSVPEQTLTIGLDGADTNDVPPTTYGWDNEKPARTVTVPAFEAQGRPITNGEYAKYLQANQSRRRPASWVLTHSDENYPIPMAVNGSSVGATQDFMSNFAVRTVFGPVPLEFAQDWPVMASYDELAEYAEWVGCRIPTFEETRSIYLHSALLKERGGVNHNGEPNGHSVNGYLNGMNGNSYSKINPGKPRTPDHQPVQYPSRDALPVFLDLDGLNVGFKHWHPTPVIQNGDRLAGQGELGGAWEWTSTPLAPHDGFKAMEIYPGYTSDFFDGKHNIILGGSWATHPRVAGRTTFVNWYQHNYPYTWAGARLVRDL

SEQ ID NO: 25 - DNA, 38 bp, Artificial sequence
  Primer
cgcaccaccttcaaaatgtcaccgttggctctttctcc

SEQ ID NO: 26 - DNA, 38 bp, Artificial sequence
  Primer
atgtactcctggtacctaaagatcccgcactaggcgtg

SEQ ID NO: 27 - DNA, 2550 bp, Artificial sequence
  Synthesized gene
gatatcatgagcccgctggcgctgagcccgaagaccgtggacattgtgaacatttttcagaacgacgtggagtttagcctggtgaacgagattcataaaggcatcagcccgccggcgggtgttcgtaaaagcatgccgaccatgctgctgtacgatgcgaacggtctgaagctgttcgaaaacattacctatgtgaaagagtactatctgaccaacgcggagatcgaagtgctggaaaccaacagccgtcgtatcgttgagcgtattccggacaacgcgcagctgctggaactgggtagcggcaacctgcgtaagatcgagattctgctgcgtgagttcgaacgtgtgggcaaacgtgttgattactatgcgctggacctgagcctgagcgaactgcaacgtacctttgcggaagtgagcattgacgattacacccacgttggtctgcacggcctgcacggtacctatgacgatgcggttacctggctgaacagcccggaaaaccgtaagcgtccgaccgtgatcatgagcatgggcagcagcctgggtaacttcgatcgtccgggtgcggcgaaatttctgagccaatatgcgagcctgctgggtccgagcgacatgatgatcattggcctggatggttgcaaggacccgggtaaagtgtaccgtgcgtataacgacagcgaaggcgttacccgtcaattctacgagaacggtctggtgcacgcgaacgtggttctgggctatgaagcgtttaagagcgatgagtgggaagtggttaccgactacgataccgttgagggtcgtcactgggcggcgtatagcccgaagaaagacgtgaccattaacggcgttctgctgaagaaaggtgaaaagctgttctttgaggaagcgtacaaatatggcccggaggaacgtgatcagctgtggcgtgacgcgaagctgatccaaagcaccgagatgggtaacggcagcgacgattaccacctgcacctgctgaccagcgcgaccctgaacctgccgaccagcccgagccagtatgcggcgcacccgattccgagcttcgaggaatggcaaagcctgtggaccgcgtgggataacgcgaccaaagcgatggttccgcgtgaggaactgctgagcaagccgatcaaactgcgtaacagcctgatcttctacctgggtcacattccgacctttctggacatccacctgacccgtgcgctgcgtggcaagctgaccgaaccgaagagctataaactgatctttgagcgtggcattgacccggatgtggacgatccggaaaaatgccacagccacagcgaaattccggatgagtggccggcgctggacgacatcctggactaccaggagcgtgtgcgtagccgtgttcgtagcatctatcaaattgaaggtctggcggagaaccgtattctgggcgaagcgctgtggatcggtttcgagcacgaagtgatgcacctggagacctttctgtacatgctgattcaaagcgaacgtatcctgccgccgccggcgaccgagcgtccggatttcaagaaactgtatcaggaagcgcgtcgtagcatgaaggcgaacgaatggtttagcgttccggagcaaaccctgaccatcggcctggacggtgcggataccaacgacgtgccgccgaccacctacggttgggacaacgaaaaaccggcgcgtaccgttaccgttccggcgtttgaagcgcagggtcgtccgattaccaacggcgagtacgcgaaatatctgcaggcgaaccaaagccgtcgtcgtccggcgagctgggttctgacccacagcgacgaagattacgcgatcccgatggcggtgaacggcagcagcgttggtgcgacccaggacttcatgagcaactttgcggtgcgtaccgttttcggtccggttccgctggagtttgcgcaagattggccggtgatggcgagctacgacgagctggcggaatatgcggagtgggtgggctgccgtattccgaccttcgaggaaacccgtagcatctacctgcacagcgcgctgctgaaggaacgtggtggcgttaaccacaacggcgagccgaacggtcacagcctgaacggcgatctgaacggtgtgaacggtaacggctacagcaaaatcaacccgggcaagccgcgtaaaccggaccaccagccggttcaatatccgagccgtgatgcgctgccggtgttcctggacctgcacggtctgaacgttggttttaaacactggcacccgaccccggtgattcagaacggtgatcgtctggcgggtcaaggtgaactgggtggcgcgtgggagtggaccagcaccccgctggcgccgcacgacggcttcaaggcgatggagatctacccgggctataccagcgatttctttgacggtaaacacaacatcattctgggtggcagctgggcgacccacccgcgtgtggcgggtcgtaccacctttgttaactggtatcaacacaattatccgtacacctgggcgggtgcgcgtctggttcgtgacctgtaaactagt

SEQ ID NO: 28 - DNA, 1404 bp, Artificial sequence
  Synthesized gene
gatatcatgaccacgccgtttggtgcgccgatgcgtgaacattttctgttcgataccaacttcaaaaacctgaatcacggttccttcggcacgtatccgcgtgcggtccagaccgtgctgcgtcagcatcaacactcagcagaagctcgcccggacctgttttatcgtattacccgcggtcaaggcatcgacggttctcgtcgcattgtcgcgaacctgctgaatatcccggtgaacgaatgcgttttcgtcaaaaatgccaccacgggcgttgcaaccgtcctgcgtaacctggtgtttcagaaaggtgatgcagtggtttatttcgacaccatctacggcgctgtggagaaaaacgttcattctattatggaagcaagtccggtcaccacgcgcaaagtggaatgtgctctgccggtttctcatgaagatctggtcaaacgttttcgcgacgtcgtgagtcgtgcgcgcggtgaaggcctgcacgtgaaagttgccgtcttcgatacgattgtgtcggttccgggcgttcgttttccgttcgaaaccctggtcggtgtgtgccgcgaagaaggcattctgagcctgatcgatggtgcgcatggtattggccacattccgctggatctgggtaccctgcgtccggactttttcacctctaacctgcataaatggctgtttgtgccgcgcggttgtgccgtgctgcatgttccgctgcgtaatcagcacctgatccgcaccacgttcccgaccagttggggttatattccgccgccgagctctggcgaaattaccccgacggcaacccagggcaaatcggcttttgaatacctgttcgaacacattagcaccacggatgatacgccgtggctgtgtgttccggccgcaatgaaatttcgtaccgaagtgtgtggcggtgaagatcgcatctatgcatacctggaaacgctggcacgtgaagctggtgacattgttgcccgtgcactgggtaccgaagtgatgcaggaaccgggtctgaaagaaggcgaagttagccaactgcgtcgctgcggtatggccaccgtgcgtctgccgatcgccgttaccagttcctcatcgagcgatagcggtagcggtaatggcggtggcgccgtcatgcgtgtgcagggtgaagacggctctagttatctgcgcattcaaacgtccctggttggcaccgtctcaaattggtttcgcgatacgctgttcgacaaatatgaaacctttgttccggtcttccagcatggtggctggctgtggacccgtctgtccgcacaagtgtacctggaaaagggtgattttgaatggctgggtggcgttctgcgcgaatgctgtgaacgtgtggaacgcgaagtgggcgtttcctcagctaaactgtaaactagt

SEQ ID NO: 29 - DNA, 2890 bp, Aspergillus niger
atgtcacccttatgtccggtcgtcaagggcgttgacatcgtcgatatccgtcaaaatgacgtggagttttccctggtaaatgatatccagcgaggtatagatcctccggcaggaacttgccgatccatgcccacaatgcttctttacgatgctcaggggctcaagctgttcgaggacattacgtacctggaggaatactatctcacaaatgcggagattgacgttctacggacacatgcgaagaggattgttgaacgcatcccggacaatgcgcaattactggaactaggcagtgggtgcgtcttccttccgcttggagcatgtatagagtatagggtacagacacgggattctaacatacggtagcaatctgcgcaagattgagatccttctccaggaattcgaagcagcgagcaaaaaagtggactactatgccttggatctgtcgctctcagagttggagcgcacattctcggaagtgtccctcgatcaatatcaatatgtcaagctccacggcctgcatggcacgtacgacgacgccctcacctggctagaaaaccccgcgaatcgaaaggtcccaacggtgatcatgtcaatgggctcgtcgataggaaattttgatcgtcctgcagcggcaaaattcttgtcgcaatttgccaggctcttagggccgtcggatttgatggtgctcggtttggatagttgcacggactcggataaagtgtacaaggcatacaatgattccaagggtatcacacggcagttctacgagaacgggttgttgcatgcgaacgctgtgcttggatacgaagcattcaaactcgatgaatgggatatcgtgacggagtacgataacgtcgaagggcggcaccaggcgttctacgcgccaaaccgggacgtgactataaacggggtactacttcagaaaggcgagaagctaatttttgaggaggcattcaaatatgatcccgagcagtgcgatcagctctggcatgatgcgggtttaattgaggacgctgagtttggcaatgagtctggggattaccgtatgtcatcctttggcaatgtgctactctgcatgtcatgttgcactgcattgtgtaaaaacatgttacaccagttgagaccatcatactaacataatctgtcgagcagttatccacgtgctctcttcggcttctctcaacttttcaacgagaccatcacagtatgcggctcaatctattccgagctttgaggaattccagtcactgtggacagcatgggacattgtcaccaaggccatggttcctagagaggaacttctttcgaagccaatcaaattgcgcaatgcattaatcttctacctcggtcacatacctacgtttctcggtcagtgttctgcttggctatttgtggagtgcaagtataggggtcagcatattgacaagcgcagatgttcatttgacccgagcattgggcgaaaagccaacgcaccccaagtcatatcgactcattttcgaacgcggaatcgaccccgatgtggatgaccccgaaaagtgccattctcacagcgagattccagacgaatggcctgcccttggagacatcttggactaccaagtgcgggttcgaagtagggtgaggtccatttttcagaagcataatgtggctgagaatagggtgcttggtgaagcactctggatcgggtttgagcatgaagccatgcatctggaaacgttcctttacatgcttatccagagtgaaagaacacttccgccccccgccgttccgcgccccgattttaggaagtttttccacgatgcccggcaagagtcaagaccaaacgagtggttttcgattcccgagaagacgctttcggttggattacatgatgatggacattcagttcctcgtgactcttttggctgggacaacgaaaagccccagagaaagataaccgttaaagcattcgaagctcaagcgcgaccaataacaaatggagagtacgcgaagtatctacaggcgaatcagctgccccagaagccagagtcctgggtcttgatcaagcccgagacgtacccgacttgcaatggtgtcagtcaagacggtagctacgctacgaatgaattcatggcacactttgccgttcgcactgtgtttggctccgtcccgctcgagctagcccaggactggccggttatcgcgtcgtacgatgaattggccaagtatgccaagtgggtggactgcaggataccaaccttcgaagaggcaaagagtatctacgcgcatgcagctcggctgaaggaaactagccacggcctgaacggtcacaggtaagcataccgcttccactagatgcacaggacttactgtcatagtgaaacgaacggagtcaacgggcacgaacatagcgagaccaaccccctacggcctcgcaccccggaccaccaaccggtacagcacccttcgcaagaatctctgccggtgtttgttgagctcgacaattgcaacgtcggcttcaaacactggcaccctaccccggtcatccagaacggcgaccgactcgccggtcatggagagctgggaggcgtctgggagtggacgagcacggaacttgcaccccacgaagggttcgaggccatgcaaatctaccccggatatacatgtaagcttgctgtgtgagatatatgaacacaagctaactgagaacagccgacttcttcgacggaaaacacaatatcatcctcggagggtcatgggcgacgcatccacggatcgccggccgcactaccttgtaagtccgtatgcaagactagcgggttcatgagctaatctgttcagtgtcaattggtaccagcggaactacccatacccctgggctggtgcccggctggtgcgggatgtctga

SEQ ID NO: 30 - protein, 835 aa, Aspergillus niger
MSPLCPVVKGVDIVDIRQNDVEFSLVNDIQRGIDPPAGTCRSMPTMLLYDAQGLKLFEDITYLEEYYLTNAEIDVLRTHAKRIVERIPDNAQLLELGSGNLRKIEILLQEFEAASKKVDYYALDLSLSELERTFSEVSLDQYQYVKLHGLHGTYDDALTWLENPANRKVPTVIMSMGSSIGNFDRPAAAKFLSQFARLLGPSDLMVLGLDSCTDSDKVYKAYNDSKGITRQFYENGLLHANAVLGYEAFKLDEWDIVTEYDNVEGRHQAFYAPNRDVTINGVLLQKGEKLIFEEAFKYDPEQCDQLWHDAGLIEDAEFGNESGDYLIHVLSSASLNFSTRPSQYAAQSIPSFEEFQSLWTAWDIVTKAMVPREELLSKPIKLRNALIFYLGHIPTFLDVHLTRALGEKPTHPKSYRLIFERGIDPDVDDPEKCHSHSEIPDEWPALGDILDYQVRVRSRVRSIFQKHNVAENRVLGEALWIGFEHEAMHLETFLYMLIQSERTLPPPAVPRPDFRKFFHDARQESRPNEWFSIPEKTLSVGLHDDGHSVPRDSFGWDNEKPQRKITVKAFEAQARPITNGEYAKYLQANQLPQKPESWVLIKPETYPTCNGVSQDGSYATNEFMAHFAVRTVFGSVPLELAQDWPVIASYDELAKYAKWVDCRIPTFEEAKSIYAHAARLKETSHGLNGHSETNGVNGHEHSETNPLRPRTPDHQPVQHPSQESLPVFVELDNCNVGFKHWHPTPVIQNGDRLAGHGELGGVWEWTSTELAPHEGFEAMQIYPGYTSDFFDGKHNIILGGSWATHPRIAGRTTFVNWYQRNYPYPWAGARLVRDV

SEQ ID NO: 31 - DNA, 42 bp, Artificial sequence
  Primer
cgcaccaccttcaaaatgtcacccttatgtccggtcgtcaag

SEQ ID NO: 32 - DNA, 35 bp, Artificial sequence
  Primer
atgtactcctggtactcagacatcccgcaccagcc